European Patent Application EP 4 748 858 A1, published May 27, 2026. Title: 靶向人源 CD7 的抗体或其抗原结合片段及其应用. Applicant: 南京蓬勃生物科技有限公司. The sequence listing filed with the application follows.

SEQUENCE LISTING (64 sequences)

SEQ ID NO: 1 - protein, 122 aa, synthetic construct
AVQLVDSGGGLVQPGGSLGLSCAASGFTFSGFDMSWYRQAPGKERMLVATITRFGGSSNYEDSVKGRFTISRDNARDTVYLQMNSLKPEDTAMYYCHAEAPAGSLWFGNNYWGQGTQVTVSS

SEQ ID NO: 2 - protein, 8 aa, synthetic construct
GFTFSGFD

SEQ ID NO: 3 - protein, 8 aa, synthetic construct
ITRFGGSS

SEQ ID NO: 4 - protein, 15 aa, synthetic construct
HAEAPAGSLWFGNNY

SEQ ID NO: 5 - protein, 122 aa, synthetic construct
AVQLVDSGGGLVQPGGSLRLSCAASGFTFSGFAMSWYRQAPGKERELVATISRFGESSNYEDSVKGRFTISRDNAKDTGYLQMNSLKPEDTAVYYCNAEAPAGSLWYGNNYWGQGTQVTVSS

SEQ ID NO: 6 - protein, 8 aa, synthetic construct
GFTFSGFA

SEQ ID NO: 7 - protein, 8 aa, synthetic construct
ISRFGESS

SEQ ID NO: 8 - protein, 15 aa, synthetic construct
NAEAPAGSLWYGNNY

SEQ ID NO: 9 - protein, 127 aa, synthetic construct
AVQLVDSGGGLVQAGGSLTLSCAASGRTFSRYTMGWFRQAPGKERELVASISWSGGSTDYADSVKDRFTISRDNTKNTVYLQMNGLKPEDTAVYYCNTDRMPYRPVVGGILSWEPYWGQGTQVTVTP

SEQ ID NO: 10 - protein, 8 aa, synthetic construct
GRTFSRYT

SEQ ID NO: 11 - protein, 8 aa, synthetic construct
ISWSGGST

SEQ ID NO: 12 - protein, 20 aa, synthetic construct
NTDRMPYRPVVGGILSWEPY

SEQ ID NO: 13 - protein, 114 aa, synthetic construct
QVKLEESGGGLVQPGGSLRLSCVASGSSFHFAFMGWYRQAPGKQRELVADISPGNSTNYADPVKGRFVISRDNAKNTVYLQMNSLKPEDTAVYFCRDLRSWGAWGRGTQVTVSS

SEQ ID NO: 14 - protein, 8 aa, synthetic construct
GSSFHFAF

SEQ ID NO: 15 - protein, 7 aa, synthetic construct
ISPGNST

SEQ ID NO: 16 - protein, 8 aa, synthetic construct
RDLRSWGA

SEQ ID NO: 17 - protein, 118 aa, synthetic construct
EVQLVESGGGLVQPGGSLRLSCASSERIFSIHAMGWYRQAPGKQRELVASITIGGSTHYADSVKGRFTISRDNAKNTVYLHMNSLKPEDTAVYYCNSMLLAGTVGGSWGQGTQVTVSS

SEQ ID NO: 18 - protein, 8 aa, synthetic construct
ERIFSIHA

SEQ ID NO: 19 - protein, 7 aa, synthetic construct
ITIGGST

SEQ ID NO: 20 - protein, 12 aa, synthetic construct
NSMLLAGTVGGS

SEQ ID NO: 21 - protein, 119 aa, synthetic construct
DVQLVESGGGLVQPGGSLRLSCAFPGSAFSFYFMGWYRQAPGKQRELVGDITPGGTANYADSVKGRFTISRDSAKNTVYLQMNSLKPEDTAVYYCNADRRVTIRPDGYWGQGTQVTVSS

SEQ ID NO: 22 - protein, 8 aa, synthetic construct
GSAFSFYF

SEQ ID NO: 23 - protein, 7 aa, synthetic construct
ITPGGTA

SEQ ID NO: 24 - protein, 13 aa, synthetic construct
NADRRVTIRPDGY

SEQ ID NO: 25 - protein, 122 aa, synthetic construct
QVQLVESGGGLVQPGGSLRLSCAASGFTFSGFDMSWYRQAPGKERELVATISRFGGSSNYEDSVKGRFTISRDNVKDTVYLQMNSLKPEDTAVYYCYALAPAGSLWHGDNYWGQGTQVTVSS

SEQ ID NO: 26 - protein, 8 aa, synthetic construct
GFTFSGFD

SEQ ID NO: 27 - protein, 8 aa, synthetic construct
ISRFGGSS

SEQ ID NO: 28 - protein, 15 aa, synthetic construct
YALAPAGSLWHGDNY

SEQ ID NO: 29 - protein, 122 aa, synthetic construct
QVKLEESGGGLVQAGGSLRLSCAAPGRTLSASIKAWFRQAPGKDREFAAAIRWSGDSTYYADSVKGRFTISRDNAKNTVDLQMNSLKPEDTAVYYCNAGGLLSNGYQPGSSWGQGTQVTVSS

SEQ ID NO: 30 - protein, 8 aa, synthetic construct
GRTLSASI

SEQ ID NO: 31 - protein, 8 aa, synthetic construct
IRWSGDST

SEQ ID NO: 32 - protein, 15 aa, synthetic construct
NAGGLLSNGYQPGSS

SEQ ID NO: 33 - protein, 113 aa, synthetic construct
AVQLVESGGGLVQPGGSLRLSCAASGFTASRDVMSWYRQPPGKERELVASIFSAGSKETYAESVKGRFTISIDNVKNTVNLQMDNLKPEDTAVYYCHRWPGYWGQGTQVTVSS

SEQ ID NO: 34 - protein, 8 aa, synthetic construct
GFTASRDV

SEQ ID NO: 35 - protein, 8 aa, synthetic construct
IFSAGSKE

SEQ ID NO: 36 - protein, 6 aa, synthetic construct
HRWPGY

SEQ ID NO: 37 - protein, 112 aa, synthetic construct
AVQLVDSGGGLVQPGGSLRLSCAASGDFARLYEMAWYRQTPGQQREVVAQITVGGSTKYADSVKGRFTISRDSAKNTVYLQMNSLRPEDTAVYYCHAWPALWGQGTQVTVSS

SEQ ID NO: 38 - protein, 8 aa, synthetic construct
GDFARLYE

SEQ ID NO: 39 - protein, 7 aa, synthetic construct
ITVGGST

SEQ ID NO: 40 - protein, 6 aa, synthetic construct
HAWPAL

SEQ ID NO: 41 - protein, 127 aa, synthetic construct
QVKLEESGGGLVQAGGSLRLSCAASGGTFNRYTMGWFRQAPGKEREFVAAISWSGGSTDYADSVKGRFTISRDNTKNTVYLQMNSLKPEDAAVYYCDTDRMPYRPVAAGILSWEANWGQGTQVTVSS

SEQ ID NO: 42 - protein, 8 aa, synthetic construct
GGTFNRYT

SEQ ID NO: 43 - protein, 8 aa, synthetic construct
ISWSGGST

SEQ ID NO: 44 - protein, 20 aa, synthetic construct
DTDRMPYRPVAAGILSWEAN

SEQ ID NO: 45 - protein, 115 aa, synthetic construct
AVQLVESGGGLVQPGGSLRLSCAASGFTFSNAVIGWYRQAPGKQRELVASITPGGRTTYPDSVKGRFIISRDNAKNTVYLEMNSLKLEDTAVYYCNDFRGLGGYWGQGTQVTVSS

SEQ ID NO: 46 - protein, 8 aa, synthetic construct
GFTFSNAV

SEQ ID NO: 47 - protein, 7 aa, synthetic construct
ITPGGRT

SEQ ID NO: 48 - protein, 9 aa, synthetic construct
NDFRGLGGY

SEQ ID NO: 49 - protein, 114 aa, synthetic construct
QVQLVESGGGLVKPGGSLRLSCAASGSSFHFAFMGWYRQAPGKQRELVADISPGNSTNYADPVKGRFTISRDNAKNSLYLQMNSLRAEDTAVYFCRDLRSWGAWGQGTLVTVSS

SEQ ID NO: 50 - protein, 118 aa, synthetic construct
EVQLVESGGGLVQPGGSLRLSCAASERIFSIHAMGWYRQAPGKQRELVSSITIGGSTHYADSVKGRFTISRDNSKNTLYLQMNSLRAEDTAVYYCNSMLLAGTVGGSWGQGTLVTVSS

SEQ ID NO: 51 - protein, 127 aa, synthetic construct
EVQLVESGGGLVQPGGSLRLSCAASGGTFNRYTMGWFRQAPGKEREFVSAISWSGGSTDYADSVKGRFTISRDNSKNTLYLQMNSLRAEDTAVYYCDTDRMPYRPVAAGILSWEANWGQGTLVTVSS

SEQ ID NO: 52 - protein, 288 aa, synthetic construct
MLLLVTSLLLCELPHPAFLLIPEVQLVESGGGLVQPGGSLRLSCAASERIFSIHAMGWYRQAPGKQRELVSSITIGGSTHYADSVKGRFTISRDNSKNTLYLQMNSLRAEDTAVYYCNSMLLAGTVGGSWGQGTLVTVSSGGGSGGGSGGGSGGGSEVQLVESGGGLVQPGGSLRLSCAASERIFSIHAMGWYRQAPGKQRELVSSITIGGSTHYADSVKGRFTISRDNSKNTLYLQMNSLRAEDTAVYYCNSMLLAGTVGGSWGQGTLVTVSSEQKLISEEDLKDEL

SEQ ID NO: 53 - protein, 22 aa, synthetic construct
MLLLVTSLLLCELPHPAFLLIP

SEQ ID NO: 54 - protein, 8 aa, synthetic construct
DYKDDDDK

SEQ ID NO: 55 - protein, 39 aa, synthetic construct
IEVMYPPPYLDNEKSNGTIIHVKGKHLCPSPLFPGPSKP

SEQ ID NO: 56 - protein, 27 aa, synthetic construct
FWVLVVVGGVLACYSLLVTVAFIIFWV

SEQ ID NO: 57 - protein, 41 aa, synthetic construct
RSKRSRLLHSDYMNMTPRRPGPTRKHYQPYAPPRDFAAYRS

SEQ ID NO: 58 - protein, 112 aa, synthetic construct
RVKFSRSADAPAYQQGQNQLYNELNLGRREEYDVLDKRRGRDPEMGGKPRRKNPQEGLYNELQKDKMAEAYSEIGMKGERRRGKGHDGLYQGLSTATKDTYDALHMQALPPR

SEQ ID NO: 59 - protein, 496 aa, synthetic construct
MLLLVTSLLLCELPHPAFLLIPQVQLVESGGGLVKPGGSLRLSCAASGSSFHFAFMGWYRQAPGKQRELVADISPGNSTNYADPVKGRFTISRDNAKNSLYLQMNSLRAEDTAVYFCRDLRSWGAWGQGTLVTVSSGGGSGGGSGGGSGGGSQVQLVESGGGLVKPGGSLRLSCAASGSSFHFAFMGWYRQAPGKQRELVADISPGNSTNYADPVKGRFTISRDNAKNSLYLQMNSLRAEDTAVYFCRDLRSWGAWGQGTLVTVSSAAADYKDDDDKIEVMYPPPYLDNEKSNGTIIHVKGKHLCPSPLFPGPSKPFWVLVVVGGVLACYSLLVTVAFIIFWVRSKRSRLLHSDYMNMTPRRPGPTRKHYQPYAPPRDFAAYRSRVKFSRSADAPAYQQGQNQLYNELNLGRREEYDVLDKRRGRDPEMGGKPRRKNPQEGLYNELQKDKMAEAYSEIGMKGERRRGKGHDGLYQGLSTATKDTYDALHMQALPPR

SEQ ID NO: 60 - protein, 504 aa, synthetic construct
MLLLVTSLLLCELPHPAFLLIPEVQLVESGGGLVQPGGSLRLSCAASERIFSIHAMGWYRQAPGKQRELVSSITIGGSTHYADSVKGRFTISRDNSKNTLYLQMNSLRAEDTAVYYCNSMLLAGTVGGSWGQGTLVTVSSGGGSGGGSGGGSGGGSEVQLVESGGGLVQPGGSLRLSCAASERIFSIHAMGWYRQAPGKQRELVSSITIGGSTHYADSVKGRFTISRDNSKNTLYLQMNSLRAEDTAVYYCNSMLLAGTVGGSWGQGTLVTVSSAAADYKDDDDKIEVMYPPPYLDNEKSNGTIIHVKGKHLCPSPLFPGPSKPFWVLVVVGGVLACYSLLVTVAFIIFWVRSKRSRLLHSDYMNMTPRRPGPTRKHYQPYAPPRDFAAYRSRVKFSRSADAPAYQQGQNQLYNELNLGRREEYDVLDKRRGRDPEMGGKPRRKNPQEGLYNELQKDKMAEAYSEIGMKGERRRGKGHDGLYQGLSTATKDTYDALHMQALPPR

SEQ ID NO: 61 - protein, 522 aa, synthetic construct
MLLLVTSLLLCELPHPAFLLIPEVQLVESGGGLVQPGGSLRLSCAASGGTFNRYTMGWFRQAPGKEREFVSAISWSGGSTDYADSVKGRFTISRDNSKNTLYLQMNSLRAEDTAVYYCDTDRMPYRPVAAGILSWEANWGQGTLVTVSSGGGSGGGSGGGSGGGSEVQLVESGGGLVQPGGSLRLSCAASGGTFNRYTMGWFRQAPGKEREFVSAISWSGGSTDYADSVKGRFTISRDNSKNTLYLQMNSLRAEDTAVYYCDTDRMPYRPVAAGILSWEANWGQGTLVTVSSAAADYKDDDDKIEVMYPPPYLDNEKSNGTIIHVKGKHLCPSPLFPGPSKPFWVLVVVGGVLACYSLLVTVAFIIFWVRSKRSRLLHSDYMNMTPRRPGPTRKHYQPYAPPRDFAAYRSRVKFSRSADAPAYQQGQNQLYNELNLGRREEYDVLDKRRGRDPEMGGKPRRKNPQEGLYNELQKDKMAEAYSEIGMKGERRRGKGHDGLYQGLSTATKDTYDALHMQALPPR

SEQ ID NO: 62 - protein, 524 aa, synthetic construct
MLLLVTSLLLCELPHPAFLLIPDVQLQESGGGLVQAGGSLRLSCAVSGYPYSSYCMGWFRQAPGKEREGVAAIDSDGRTRYADSVKGRFTISQDNAKNTLYLQMNRMKPEDTAMYYCAARFGPMGCVDLSTLSFGHWGQGTQVTVSITGGGGSGGGGSGGGGSGGGGSDVQLQESGGGLVQAGGSLRLSCAVSGYPYSSYCMGWFRQAPGKEREGVAAIDSDGRTRYADSVKGRFTISQDNAKNTLYLQMNRMKPEDTAMYYCAARFGPMGCVDLSTLSFGHWGQGTQVTVSITAAADYKDDDDKIEVMYPPPYLDNEKSNGTIIHVKGKHLCPSPLFPGPSKPFWVLVVVGGVLACYSLLVTVAFIIFWVRSKRSRLLHSDYMNMTPRRPGPTRKHYQPYAPPRDFAAYRSRVKFSRSADAPAYQQGQNQLYNELNLGRREEYDVLDKRRGRDPEMGGKPRRKNPQEGLYNELQKDKMAEAYSEIGMKGERRRGKGHDGLYQGLSTATKDTYDALHMQALPPR

SEQ ID NO: 63 - protein, 14 aa, synthetic construct
EQKLISEEDLKDEL

SEQ ID NO: 64 - protein, 16 aa, synthetic construct
GGGSGGGSGGGSGGGS